European Patent Specification EP 3 615 066 B1, published December 27, 2023. Title: FORMULATIONS OF HUMAN ANTI-RANKL ANTIBODIES, AND METHODS OF USING THE SAME. Applicant: Amgen Inc. The sequence listing filed with the application follows.

SEQUENCE LISTING (27 sequences)

SEQ ID NO: 1 - protein, 108 aa, Homo sapiens
  MISC_FEATURE: denosumab variable light chain
EIVLTQSPGTLSLSPGERATLSCRASQSVRGRYLAWYQQKPGQAPRLLIYGASSRATGIPDRFSGSGSGTDFTLTISRLEPEDFAVFYCQQYGSSPRTFGQGTKVEIK

SEQ ID NO: 2 - protein, 122 aa, Homo sapiens
  MISC_FEATURE: denosumab variable heavy chain
EVQLLESGGGLVQPGGSLRLSCAASGFTFSSYAMSWVRQAPGKGLEWVSGITGSGGSTYYADSVKGRFTISRDNSKNTLYLQMNSLRAEDTAVYYCAKDPGTTVIMSWFDPWGQGTLVTVSS

SEQ ID NO: 3 - protein, 235 aa, Homo sapiens
  MISC_FEATURE: denosumab full length light chain
METPAQLLFLLLLWLPDTTGEIVLTQSPGTLSLSPGERATLSCRASQSVRGRYLAWYQQKPGQAPRLLIYGASSRATGIPDRFSGSGSGTDFTLTISRLEPEDFAVFYCQQYGSSPRTFGQGTKVEIKRTVAAPSVFIFPPSDEQLKSGTASVVCLLNNFYPREAKVQWKVDNALQSGNSQESVTEQDSKDSTYSLSSTLTLSKADYEKHKVYACEVTHQGLSSPVTKSFNRGEC

SEQ ID NO: 4 - protein, 467 aa, Homo sapiens
  MISC_FEATURE: denosumab full length heavy chain
MEFGLSWLFLVAILKGVQCEVQLLESGGGLVQPGGSLRLSCAASGFTFSSYAMSWVRQAPGKGLEWVSGITGSGGSTYYADSVKGRFTISRDNSKNTLYLQMNSLRAEDTAVYYCAKDPGTTVIMSWFDPWGQGTLVTVSSASTKGPSVFPLAPCSRSTSESTAALGCLVKDYFPEPVTVSWNSGALTSGVHTFPAVLQSSGLYSLSSVVTVPSSNFGTQTYTCNVDHKPSNTKVDKTVERKCCVECPPCPAPPVAGPSVFLFPPKPKDTLMISRTPEVTCVVVDVSHEDPEVQFNWYVDGVEVHNAKTKPREEQFNSTFRVVSVLTVVHQDWLNGKEYKCKVSNKGLPAPIEKTISKTKGQPREPQVYTLPPSREEMTKNQVSLTCLVKGFYPSDIAVEWESNGQPENNYKTTPPMLDSDGSFFLYSKLTVDKSRWQQGNVFSCSVMHEALHNHYTQKSLSLSPGK

SEQ ID NO: 5 - protein, 12 aa, Homo sapiens
  MISC_FEATURE: Light Chain CDR 1
RASQSVRGRYLA

SEQ ID NO: 6 - protein, 7 aa, Homo sapiens
  MISC_FEATURE: Light Chain CDR 2
GASSRAT

SEQ ID NO: 7 - protein, 9 aa, Homo sapiens
  MISC_FEATURE: Light Chain CDR 3
QQYGSSPRT

SEQ ID NO: 8 - protein, 5 aa, Homo sapiens
  MISC_FEATURE: Heavy Chain CDR 1
SYAMS

SEQ ID NO: 9 - protein, 17 aa, Homo sapiens
  MISC_FEATURE: Heavy Chain CDR 2
GITGSGGSTYYADSVKG

SEQ ID NO: 10 - protein, 13 aa, Homo sapiens
  MISC_FEATURE: Heavy Chain CDR 3
DPGTTVIMSWFDP

SEQ ID NO: 11 - DNA, 2141 bp, Homo sapiens
ggccaaagccgggctccaagtcggcgccccacgtcgaggctccgccgcagcctccggagttggccgcagacaagaaggggagggagcgggagagggaggagagctccgaagcgagagggccgagcgccatgcgccgcgccagcagagactacaccaagtacctgcgtggctcggaggagatgggcggcggccccggagccccgcacgagggccccctgcacgccccgccgccgcctgcgccgcaccagccccccgccgcctcccgctccatgttcgtggccctcctggggctggggctgggccaggttgtctgcagcgtcgccctgttcttctatttcagagcgcagatggatcctaatagaatatcagaagatggcactcactgcatttatagaattttgagactccatgaaaatgcagattttcaagacacaactctggagagtcaagatacaaaattaatacctgattcatgtaggagaattaaacaggcctttcaaggagctgtgcaaaaggaattacaacatatcgttggatcacagcacatcagagcagagaaagcgatggtggatggctcatggttagatctggccaagaggagcaagcttgaagctcagccttttgctcatctcactattaatgccaccgacatcccatctggttcccataaagtgagtctgtcctcttggtaccatgatcggggttgggccaagatctccaacatgacttttagcaatggaaaactaatagttaatcaggatggcttttattacctgtatgccaacatttgctttcgacatcatgaaacttcaggagacctagctacagagtatcttcaactaatggtgtacgtcactaaaaccagcatcaaaatcccaagttctcataccctgatgaaaggaggaagcaccaagtattggtcagggaattctgaattccatttttattccataaacgttggtggattttttaagttacggtctggagaggaaatcagcatcgaggtctccaacccctccttactggatccggatcaggatgcaacatactttggggcttttaaagttcgagatatagattgagccccagtttttggagtgttatgtatttcctggatgtttggaaacattttttaaaacaagccaagaaagatgtatataggtgtgtgagactactaagaggcatggccccaacggtacacgactcagtatccatgctcttgaccttgtagagaacacgcgtatttacctgccagtgggagatgttagactcatggtgtgttacacaatggtttttaaattttgtaatgaattcctagaattaaaccagattggagcaattacgggttgaccttatgagaaactgcatgtgggctatgggaggggttggtccctggtcatgtgccccttcgcagctgaagtggagagggtgtcatctagcgcaattgaaggatcatctgaaggggcaaattcttttgaattgttacatcatgctggaacctgcaaaaaatactttttctaatgaggagagaaaatatatgtatttttatataatatctaaagttatatttcagatgtaatgttttctttgcaaagtattgtaaattatatttgtgctataacagacatatttaactggtgcactttgtaaattccctggggaaaacttgcagctaaggaggggaaaaaaatgttgtttcctaatatcaaatgcagtatatttcttcgttctttttaagttaatagattttttcagacttgtcaagcctgtgcaaaaaaattaaaatggatgccttgaataataagcaggatgttggccaccaggtgcctttcaaatttagaaactaattgactttagaaagctgacattgccaaaaaggatacataatgggccactgaaatttgtcaagagtagttatataattgttgaacaggtgtttttccacaagtgccgcaaattgtacctttttttttttttcaaaatagaaaagttattagtggtttatcagcaaaaaagtccaattttaatttagtaaatgttattttatactgtacaataaaaacattgcctttgaatgttaattttttggtacaaaaataaatttatatgaaaaaaaaaaaaaaaaaaaaaaaaaaaaaaaa

SEQ ID NO: 12 - protein, 317 aa, Homo sapiens
MRRASRDYTKYLRGSEEMGGGPGAPHEGPLHAPPPPAPHQPPAASRSMFVALLGLGLGQVVCSVALFFYFRAQMDPNRISEDGTHCIYRILRLHENADFQDTTLESQDTKLIPDSCRRIKQAFQGAVQKELQHIVGSQHIRAEKAMVDGSWLDLAKRSKLEAQPFAHLTINATDIPSGSHKVSLSSWYHDRGWAKISNMTFSNGKLIVNQDGFYYLYANICFRHHETSGDLATEYLQLMVYVTKTSIKIPSSHTLMKGGSTKYWSGNSEFHFYSINVGGFFKLRSGEEISIEVSNPSLLDPDQDATYFGAFKVRDID

SEQ ID NO: 13 - protein, 215 aa, Artificial Sequence
  Synthetic Polypeptide
EIVLTQSPGTLSLSPGERATLSCRASQSVRGRYLAWYQQKPGQAPRLLIYGASSRATGIPDRFSGSGSGTDFTLTISRLEPEDFAVFYCQQYGSSPRTFGQGTKVEIKRTVAAPSVFIFPPSDEQLKSGTASVVCLLNNFYPREAKVQWKVDNALQSGNSQESVTEQDSKDSTYSLSSTLTLSKADYEKHKVYACEVTHQGLSSPVTKSFNRGEC

SEQ ID NO: 14 - protein, 448 aa, Artificial Sequence
  Synthetic Polypeptide
EVQLLESGGGLVQPGGSLRLSCAASGFTFSSYAMSWVRQAPGKGLEWVSGITGSGGSTYYADSVKGRFTISRDNSKNTLYLQMNSLRAEDTAVYYCAKDPGTTVIMSWFDPWGQGTLVTVSSASTKGPSVFPLAPCSRSTSESTAALGCLVKDYFPEPVTVSWNSGALTSGVHTFPAVLQSSGLYSLSSVVTVPSSNFGTQTYTCNVDHKPSNTKVDKTVERKCCVECPPCPAPPVAGPSVFLFPPKPKDTLMISRTPEVTCVVVDVSHEDPEVQFNWYVDGVEVHNAKTKPREEQFNSTFRVVSVLTVVHQDWLNGKEYKCKVSNKGLPAPIEKTISKTKGQPREPQVYTLPPSREEMTKNQVSLTCLVKGFYPSDIAVEWESNGQPENNYKTTPPMLDSDGSFFLYSKLTVDKSRWQQGNVFSCSVMHEALHNHYTQKSLSLSPGK

SEQ ID NO: 15 - protein, 330 aa, Artificial Sequence
  Synthetic Polypeptide
  misc_feature (14)..(14): Xaa is Cys or Ser
  misc_feature (16)..(16): Xaa is Arg or Lys
  misc_feature (20)..(20): Xaa is Glu or Gly
  misc_feature (21)..(21): Xaa is Ser or Gly
  misc_feature (75)..(75): Xaa is Ser or Asn
  misc_feature (76)..(76): Xaa is Leu or Phe
  misc_feature (79)..(79): Xaa is Lys or Gln
  misc_feature (82)..(82): Xaa is Thr or Ile
  misc_feature (86)..(86): Xaa is Asp or Asn
  misc_feature (97)..(97): Xaa is Arg, Thr, or Lys
  misc_feature (100)..(100): Xaa is Ser, Arg, or Pro
  misc_feature (102)..(102): Xaa is Tyr, Cys, or Ser
  misc_feature (103)..(103): Xaa is Gly or Cys
  misc_feature (104)..(104): Xaa is absent or Asp
  misc_feature (105)..(105): Xaa is absent or Lys
  misc_feature (106)..(106): Xaa is absent or Thr
  misc_feature (107)..(107): Xaa is Pro, Val or His
  misc_feature (108)..(108): Xaa is Pro, Glu, or Thr
  misc_feature (111)..(111): Xaa is Ser or Pro
  misc_feature (116)..(116): Xaa is Glu or Pro
  misc_feature (117)..(117): Xaa is Phe, Val, or Leu
  misc_feature (118)..(118): Xaa is Leu or Ala
  misc_feature (120)..(120): Xaa is absent or Gly
  misc_feature (151)..(151): Xaa is Gln or His
  misc_feature (157)..(157): Xaa is Gln or Lys
  misc_feature (179)..(179): Xaa is Phe or Tyr
  misc_feature (183)..(183): Xaa is Tyr or Phe
  misc_feature (192)..(192): Xaa is Leu or Val
  misc_feature (210)..(210): Xaa is Gly or Ala
  misc_feature (213)..(213): Xaa is Ser or Ala
  misc_feature (214)..(214): Xaa is Ser or Pro
  misc_feature (222)..(222): Xaa is Ala or Thr
  misc_feature (238)..(238): Xaa is Gln or Arg
  misc_feature (239)..(239): Xaa is Glu or Asp
  misc_feature (241)..(241): Xaa is Met or Leu
  misc_feature (280)..(280): Xaa is Val or Met
  misc_feature (292)..(292): Xaa is Arg or Lys
  misc_feature (302)..(302): Xaa is Glu or Gln
  misc_feature (328)..(328): Xaa is Leu or Pro
ASTKGPSVFPLAPXSXSTSXXTAALGCLVKDYFPEPVTVSWNSGALTSGVHTFPAVLQSSGLYSLSSVVTVPSSXXGTXTYXCNVXHKPSNTKVDKXVEXKXXXXXXXCPXCPAPXXXGXPSVFLFPPKPKDTLMISRTPEVTCVVVDVSXEDPEVXFNWYVDGVEVHNAKTKPREEQXNSTXRVVSVLTVXHQDWLNGKEYKCKVSNKXLPXXIEKTISKXKGQPREPQVYTLPPSXXEXTKNQVSLTCLVKGFYPSDIAVEWESNGQPENNYKTTPPXLDSDGSFFLYSXLTVDKSRWQXGNVFSCSVMHEALHNHYTQKSLSLSXGK

SEQ ID NO: 16 - protein, 326 aa, Artificial Sequence
  Synthetic Polypeptide
  MISC_FEATURE: IgG2 Constant HC
ASTKGPSVFPLAPCSRSTSESTAALGCLVKDYFPEPVTVSWNSGALTSGVHTFPAVLQSSGLYSLSSVVTVPSSNFGTQTYTCNVDHKPSNTKVDKTVERKCCVECPPCPAPPVAGPSVFLFPPKPKDTLMISRTPEVTCVVVDVSHEDPEVQFNWYVDGVEVHNAKTKPREEQFNSTFRVVSVLTVVHQDWLNGKEYKCKVSNKGLPAPIEKTISKTKGQPREPQVYTLPPSREEMTKNQVSLTCLVKGFYPSDIAVEWESNGQPENNYKTTPPMLDSDGSFFLYSKLTVDKSRWQQGNVFSCSVMHEALHNHYTQKSLSLSPGK

SEQ ID NO: 17 - protein, 330 aa, Artificial Sequence [sequence omitted]

SEQ ID NO: 18 - protein, 327 aa, Artificial Sequence
  Synthetic Polypeptide
  MISC_FEATURE: IgG4 constant HC
ASTKGPSVFPLAPCSRSTSESTAALGCLVKDYFPEPVTVSWNSGALTSGVHTFPAVLQSSGLYSLSSVVTVPSSSLGTKTYTCNVDHKPSNTKVDKRVESKYGPPCPSCPAPEFLGGPSVFLFPPKPKDTLMISRTPEVTCVVVDVSQEDPEVQFNWYVDGVEVHNAKTKPREEQFNSTYRVVSVLTVLHQDWLNGKEYKCKVSNKGLPSSIEKTISKAKGQPREPQVYTLPPSQEEMTKNQVSLTCLVKGFYPSDIAVEWESNGQPENNYKTTPPVLDSDGSFFLYSRLTVDKSRWQEGNVFSCSVMHEALHNHYTQKSLSLSLGK

SEQ ID NO: 19 - DNA, 324 bp, Artificial Sequence
  Synthetic Polynucleotide
  misc_feature: variable LC
gaaattgtgttgacgcagtctccaggcaccctgtctttgtctccaggggaaagagccaccctctcctgtagggccagtcagagtgttcgcggcaggtacttagcctggtaccagcagaaacctggccaggctcccaggctcctcatctatggtgcatccagcagggccactggcatcccagacaggttcagtggcagtgggtctgggacagacttcactctcaccatcagcagactggagcctgaagattttgcagtgttttactgtcagcagtatggtagttcacctcggacgttcggccaagggaccaaggtggaaatcaaa

SEQ ID NO: 20 - DNA, 366 bp, Artificial Sequence
  Synthetic Polynucleotide
  misc_feature: variable HC
gaggtgcagctgttggagtctgggggaggcttggtacagcctggggggtccctgagactctcctgtgcagcctctggattcacctttagcagctatgccatgagctgggtccgccaggctccagggaaggggctggagtgggtctcaggtattactgggagtggtggtagtacatactacgcagactccgtgaagggccggttcaccatctccagagacaattccaagaacacgctgtatctgcaaatgaacagcctgagagccgaggacacggccgtatattactgtgcgaaagatccagggactacggtgattatgagttggttcgacccctggggccagggaaccctggtcaccgtctcctca

SEQ ID NO: 21 - DNA, 705 bp, Artificial Sequence
  Synthetic Polynucleotide
  misc_feature: full length LC
atggaaaccccagcgcagcttctcttcctcctgctactctggctcccagataccaccggagaaattgtgttgacgcagtctccaggcaccctgtctttgtctccaggggaaagagccaccctctcctgtagggccagtcagagtgttcgcggcaggtacttagcctggtaccagcagaaacctggccaggctcccaggctcctcatctatggtgcatccagcagggccactggcatcccagacaggttcagtggcagtgggtctgggacagacttcactctcaccatcagcagactggagcctgaagattttgcagtgttttactgtcagcagtatggtagttcacctcggacgttcggccaagggaccaaggtggaaatcaaacgaactgtggctgcaccatctgtcttcatcttcccgccatctgatgagcagttgaaatctggaactgcctctgttgtgtgcctgctgaataacttctatcccagagaggccaaagtacagtggaaggtggataacgccctccaatcgggtaactcccaggagagtgtcacagagcaggacagcaaggacagcacctacagcctcagcagcaccctgacgctgagcaaagcagactacgagaaacacaaagtctacgcctgcgaagtcacccatcagggcctgagctcgcccgtcacaaagagcttcaacaggggagagtgt

SEQ ID NO: 22 - DNA, 1401 bp, Artificial Sequence
  Synthetic Polynucleotide
  misc_feature: full length HC
atggagtttgggctgagctggctttttcttgtggctattttaaaaggtgtccagtgtgaggtgcagctgttggagtctgggggaggcttggtacagcctggggggtccctgagactctcctgtgcagcctctggattcacctttagcagctatgccatgagctgggtccgccaggctccagggaaggggctggagtgggtctcaggtattactgggagtggtggtagtacatactacgcagactccgtgaagggccggttcaccatctccagagacaattccaagaacacgctgtatctgcaaatgaacagcctgagagccgaggacacggccgtatattactgtgcgaaagatccagggactacggtgattatgagttggttcgacccctggggccagggaaccctggtcaccgtctcctcagcctccaccaagggcccatcggtcttccccctggcgccctgctccaggagcacctccgagagcacagcggccctgggctgcctggtcaaggactacttccccgaaccggtgacggtgtcgtggaactcaggcgctctgaccagcggcgtgcacaccttcccagctgtcctacagtcctcaggactctactccctcagcagcgtggtgaccgtgccctccagcaacttcggcacccagacctacacctgcaacgtagatcacaagcccagcaacaccaaggtggacaagacagttgagcgcaaatgttgtgtcgagtgcccaccgtgcccagcaccacctgtggcaggaccgtcagtcttcctcttccccccaaaacccaaggacaccctcatgatctcccggacccctgaggtcacgtgcgtggtggtggacgtgagccacgaagaccccgaggtccagttcaactggtacgtggacggcgtggaggtgcataatgccaagacaaagccacgggaggagcagttcaacagcacgttccgtgtggtcagcgtcctcaccgttgtgcaccaggactggctgaacggcaaggagtacaagtgcaaggtctccaacaaaggcctcccagcccccatcgagaaaaccatctccaaaaccaaagggcagccccgagaaccacaggtgtacaccctgcccccatcccgggaggagatgaccaagaaccaggtcagcctgacctgcctggtcaaaggcttctaccccagcgacatcgccgtggagtgggagagcaatgggcagccggagaacaactacaagaccacacctcccatgctggactccgacggctccttcttcctctacagcaagctcaccgtggacaagagcaggtggcagcaggggaacgtcttctcatgctccgtgatgcatgaggctctgcacaaccactacacgcagaagagcctctccctgtctccgggtaaa

SEQ ID NO: 23 - DNA, 645 bp, Artificial Sequence
  Synthetic Polynucleotide
  misc_feature: mature LC
gaaattgtgttgacgcagtctccaggcaccctgtctttgtctccaggggaaagagccaccctctcctgtagggccagtcagagtgttcgcggcaggtacttagcctggtaccagcagaaacctggccaggctcccaggctcctcatctatggtgcatccagcagggccactggcatcccagacaggttcagtggcagtgggtctgggacagacttcactctcaccatcagcagactggagcctgaagattttgcagtgttttactgtcagcagtatggtagttcacctcggacgttcggccaagggaccaaggtggaaatcaaacgaactgtggctgcaccatctgtcttcatcttcccgccatctgatgagcagttgaaatctggaactgcctctgttgtgtgcctgctgaataacttctatcccagagaggccaaagtacagtggaaggtggataacgccctccaatcgggtaactcccaggagagtgtcacagagcaggacagcaaggacagcacctacagcctcagcagcaccctgacgctgagcaaagcagactacgagaaacacaaagtctacgcctgcgaagtcacccatcagggcctgagctcgcccgtcacaaagagcttcaacaggggagagtgt

SEQ ID NO: 24 - DNA, 1344 bp, Artificial Sequence
  Synthetic Polynucleotide
  misc_feature: mature HC
gaggtgcagctgttggagtctgggggaggcttggtacagcctggggggtccctgagactctcctgtgcagcctctggattcacctttagcagctatgccatgagctgggtccgccaggctccagggaaggggctggagtgggtctcaggtattactgggagtggtggtagtacatactacgcagactccgtgaagggccggttcaccatctccagagacaattccaagaacacgctgtatctgcaaatgaacagcctgagagccgaggacacggccgtatattactgtgcgaaagatccagggactacggtgattatgagttggttcgacccctggggccagggaaccctggtcaccgtctcctcagcctccaccaagggcccatcggtcttccccctggcgccctgctccaggagcacctccgagagcacagcggccctgggctgcctggtcaaggactacttccccgaaccggtgacggtgtcgtggaactcaggcgctctgaccagcggcgtgcacaccttcccagctgtcctacagtcctcaggactctactccctcagcagcgtggtgaccgtgccctccagcaacttcggcacccagacctacacctgcaacgtagatcacaagcccagcaacaccaaggtggacaagacagttgagcgcaaatgttgtgtcgagtgcccaccgtgcccagcaccacctgtggcaggaccgtcagtcttcctcttccccccaaaacccaaggacaccctcatgatctcccggacccctgaggtcacgtgcgtggtggtggacgtgagccacgaagaccccgaggtccagttcaactggtacgtggacggcgtggaggtgcataatgccaagacaaagccacgggaggagcagttcaacagcacgttccgtgtggtcagcgtcctcaccgttgtgcaccaggactggctgaacggcaaggagtacaagtgcaaggtctccaacaaaggcctcccagcccccatcgagaaaaccatctccaaaaccaaagggcagccccgagaaccacaggtgtacaccctgcccccatcccgggaggagatgaccaagaaccaggtcagcctgacctgcctggtcaaaggcttctaccccagcgacatcgccgtggagtgggagagcaatgggcagccggagaacaactacaagaccacacctcccatgctggactccgacggctccttcttcctctacagcaagctcaccgtggacaagagcaggtggcagcaggggaacgtcttctcatgctccgtgatgcatgaggctctgcacaaccactacacgcagaagagcctctccctgtctccgggtaaa

SEQ ID NO: 25 - protein, 20 aa, Artificial Sequence
  Synthetic Polypeptide
  MISC_FEATURE: signal peptide of full length LC of SEQ 3
METPAQLLFLLLLWLPDTTG

SEQ ID NO: 26 - protein, 19 aa, Artificial Sequence
  Synthetic Polypeptide
  MISC_FEATURE: signal peptide of full length HC of SEQ 4
MEFGLSWLFLVAILKGVQC

SEQ ID NO: 27 - protein, 10 aa, Artificial Sequence
  Synthetic Polypeptide
GFTFSSYAMS